European Patent Application EP 4 166 571 A1, published April 19, 2023. Title: ANTIBODIES BINDING CD70, PREPARATION AND USE THEREOF. Applicant: ImmuneOnco Biopharmaceuticals (Shanghai) Co., Ltd. The sequence listing filed with the application follows.

SEQUENCE LISTING (23 sequences)

SEQ ID NO: 1 - protein, 8 aa, Artificial Sequence
  HV-CDR1 of IMM40C, IMM40H and IMM40M
GYTFTDSA

SEQ ID NO: 2 - protein, 8 aa, Artificial Sequence
  HV-CDR2 of IMM40C, IMM40H and IMM40M
ISTYDGDT

SEQ ID NO: 3 - protein, 13 aa, Artificial Sequence
  HV-CDR3 of IMM40C, IMM40H and IMM40M
ARRGYYDYDWFPY

SEQ ID NO: 4 - protein, 10 aa, Artificial Sequence
  LV-CDR1 of IMM40C, IMM40H and IMM40M
KSVSASGYSF

SEQ ID NO: 5 - protein, 3 aa, Artificial Sequence
  LV-CDR2 of IMM40C, IMM40H and IMM40M
LAS

SEQ ID NO: 6 - protein, 9 aa, Artificial Sequence
  LV-CDR3 of IMM40C, IMM40H and IMM40M
QHSRELPPT

SEQ ID NO: 7 - protein, 120 aa, Artificial Sequence
  Heavy chain variable region of IMM40C
QVQLQQSGPEVVRPGVSVKISCKGSGYTFTDSALHWVKQSHAKSLEWIGVISTYDGDTDYNQKFKGKATMTVDKSSSTAYMELARLTSEDSAIYYCARRGYYDYDWFPYWGQGTLVTVSA

SEQ ID NO: 8 - protein, 111 aa, Artificial Sequence
  Light chain variable region of IMM40C
DIVLTQSPASLAISLGQRATISCRASKSVSASGYSFLHWYQQKPGQPPKLLIYLASNLESGVPARFSGSGSGTDFTLNIHPVEEEDAATFYCQHSRELPPTFGGGTKLEIK

SEQ ID NO: 9 - protein, 120 aa, Artificial Sequence
  Heavy chain variable region of IMM40H and IMM40M
QVQLVQSGAEVKKPGASVKVSCKVSGYTFTDSALHWVRQAPGKGLEWMGVISTYDGDTDYNQKFKGRVTMTEDTSTDTAYMELSSLRSEDTAVYYCARRGYYDYDWFPYWGQGTLVTVSA

SEQ ID NO: 10 - protein, 111 aa, Artificial Sequence
  Light chain variable region of IMM40H/IMM40M
  misc_feature (85)..(85): Xaa can be Asn or Glu
DIVLTQSPASLAVSPGQRATITCRASKSVSASGYSFLHWYQQKPGQPPKLLIYLASNLESGVPARFSGSGSGTDFTLTINPVEAXDTANYYCQHSRELPPTFGGGTKVEIK

SEQ ID NO: 11 - protein, 330 aa, Artificial Sequence
  Heavy chain constant region
ASTKGPSVFPLAPSSKSTSGGTAALGCLVKDYFPEPVTVSWNSGALTSGVHTFPAVLQSSGLYSLSSVVTVPSSSLGTQTYICNVNHKPSNTKVDKRVEPKSCDKTHTCPPCPAPELLGGPSVFLFPPKPKDTLMISRTPEVTCVVVDVSHEDPEVKFNWYVDGVEVHNAKTKPREEQYNATYRVVSVLTVLHQDWLNGKEYKCKVSNKALPAPIAATISKAKGQPREPQVYTLPPSREEMTKNQVSLTCLVKGFYPSDIAVEWESNGQPENNYKTTPPVLDSDGSFFLYSKLTVDKSRWQQGNVFSCSVMHEALHNHYTQKSLSLSPGK

SEQ ID NO: 12 - protein, 107 aa, Artificial Sequence [sequence omitted]

SEQ ID NO: 13 - DNA, 1410 bp, Artificial Sequence
  IMM40C's heavy chain
atgggttggagctgtatcatcttctttctggtagcaacagctacaggtgtgcactcccaggtccagctgcagcagtctgggcctgaggtggtgaggcctggggtctcagtgaagatttcctgcaagggttccggctacacattcactgatagtgctttgcactgggtgaagcagagtcatgcaaagagtctagagtggattggagttattagtacttacgatggtgatacagactacaaccagaagtttaagggcaaggccacaatgactgtagacaaatcctccagcacagcctatatggaacttgccagattgacatctgaggattctgccatctattactgtgcaagaaggggatactatgattacgactggtttccttactggggccaagggactctggtcactgtctctgcagctagcaccaagggcccatcggtcttccccctggcaccctcctccaagagcacctctgggggcacagcggccctgggctgcctggtcaaggactacttccccgaaccggtgacggtgtcgtggaactcaggcgccctgaccagcggcgtgcacaccttcccggctgtcctacagtcctcaggactctactccctcagcagcgtggtgaccgtgccctccagcagcttgggcacccagacctacatctgcaacgtgaatcacaagcccagcaacaccaaggtggacaagagagttgagcccaaatcttgtgacaaaactcacacatgcccaccgtgcccagcacctgaactcctggggggaccgtcagtcttcctcttccccccaaaacccaaggacaccctcatgatctcccggacccctgaggtcacatgcgtggtggtggacgtgagccacgaagaccctgaggtcaagttcaactggtatgtggacggcgtggaggtgcataatgccaagacaaagccgcgggaggagcagtacaacgccacgtaccgtgtggtcagcgtcctcaccgtcctgcaccaagactggctgaatggcaaggagtacaagtgcaaggtctccaacaaagccctcccagcccccatcgccgcaaccatctccaaagccaaagggcagccccgagaaccacaggtgtacaccctgcccccatcccgggaggagatgaccaagaaccaagtcagcctgacctgcctggtcaaaggcttctatcccagcgacatcgccgtggagtgggagagcaatgggcagccggagaacaactacaagaccacgcctcccgtgctggactccgacggctccttcttcctctattccaagctcaccgtggacaagagcaggtggcagcaggggaacgtcttctcatgctccgtgatgcatgaggctctgcacaaccactacacgcagaagagcctctccctgtctccgggcaaatga

SEQ ID NO: 14 - DNA, 856 bp, Artificial Sequence
  IMM40C's light chain
atggagacagacacactcctgttatgggtactgctgctctgggttccaggttccactggtgacattgtgctgacacagtctcctgcttccttagctatatctctggggcagagggccaccatctcatgcagggccagcaaaagtgtcagtgcatctggctatagttttctgcactggtaccaacagaaaccaggacagccacccaaactcctcatctatcttgcatccaacctcgaatctggggtccctgccaggttcagtggcagtgggtctgggacagactttaccctcaacatccatcctgtggaggaggaggatgctgcaaccttttactgtcagcacagtagggagcttcctccgacgttcggtggaggcaccaaactggaaatcaaacgtgagttctagaggatccatctgggataagcatgctgttttctgtctgtccctaacatgccctgtgattatccgcaaacaacacacccaagggcagaactttgttacttaaacaccatcctgtttgcttctttcctcaggaactgtggctgcaccatctgtcttcatcttcccgccatctgatgagcagttgaaatctggaactgcctctgttgtgtgcctgctgaataacttctatcccagagaggccaaagtacagtggaaggtggataacgccctccaatcgggtaactcccaggagagtgtcacagagcaggacagcaaggacagcacctacagcctcagcagcaccctgacgctgagcaaagcagactacgagaaacacaaagtctacgcctgcgaagtcacccatcagggcctgagctcgcccgtcacaaagagcttcaacaggggagagtgttag

SEQ ID NO: 15 - DNA, 1410 bp, Artificial Sequence
  IMM40H/IMM40M's heavy chain
atgggatggtcatgtatcatcctttttctggtagcaactgcaactggagtacattcacaagtgcagctggtgcagagcggcgccgaggtgaagaagcctggcgcaagcgtgaaggtgagctgcaaggtgagcggctacaccttcaccgacagcgccctgcactgggtgagacaagcccctggcaagggcctggagtggatgggcgtgatcagcacctacgacggcgacaccgactacaatcagaagttcaagggcagagtgaccatgaccgaggacacaagcaccgacaccgcctacatggagctgagcagcctgagaagcgaggacaccgccgtgtactactgcgctagaagaggctactacgactacgactggttcccttactggggccaaggcaccctggtgaccgtgagcgccgctagcaccaagggcccatcggtcttccccctggcaccctcctccaagagcacctctgggggcacagcggccctgggctgcctggtcaaggactacttccccgaaccggtgacggtgtcgtggaactcaggcgccctgaccagcggcgtgcacaccttcccggctgtcctacagtcctcaggactctactccctcagcagcgtggtgaccgtgccctccagcagcttgggcacccagacctacatctgcaacgtgaatcacaagcccagcaacaccaaggtggacaagagagttgagcccaaatcttgtgacaaaactcacacatgcccaccgtgcccagcacctgaactcctggggggaccgtcagtcttcctcttccccccaaaacccaaggacaccctcatgatctcccggacccctgaggtcacatgcgtggtggtggacgtgagccacgaagaccctgaggtcaagttcaactggtatgtggacggcgtggaggtgcataatgccaagacaaagccgcgggaggagcagtacaacgccacgtaccgtgtggtcagcgtcctcaccgtcctgcaccaagactggctgaatggcaaggagtacaagtgcaaggtctccaacaaagccctcccagcccccatcgccgcaaccatctccaaagccaaagggcagccccgagaaccacaggtgtacaccctgcccccatcccgggaggagatgaccaagaaccaagtcagcctgacctgcctggtcaaaggcttctatcccagcgacatcgccgtggagtgggagagcaatgggcagccggagaacaactacaagaccacgcctcccgtgctggactccgacggctccttcttcctctattccaagctcaccgtggacaagagcaggtggcagcaggggaacgtcttctcatgctccgtgatgcatgaggctctgcacaaccactacacgcagaagagcctctccctgtctccgggcaaatga

SEQ ID NO: 16 - DNA, 853 bp, Artificial Sequence
  IMM40H/IMM40M's light chain
  misc_feature (310)..(310): n is a or g
  misc_feature (312)..(312): n is c or a
atgggatggtcatgtatcatcctttttctggtagcaactgcaactggagtacattcagacatcgtgctgacacagagccctgcaagcctggccgtgagccctggacagagagccaccatcacctgcagagcaagcaagagcgtgagcgcaagcggctacagcttcctgcactggtatcagcagaagcctggacagcctcctaagctgctgatctacctggcaagcaacctggagagcggcgtgcctgctagattcagcggcagcggcagcggcaccgacttcaccctgaccatcaaccctgtggaggccnangacaccgccaactactactgtcagcacagcagagagctgcctcctaccttcggcggcggcaccaaggtggagatcaagcgtgagttctagaggatccatctgggataagcatgctgttttctgtctgtccctaacatgccctgtgattatccgcaaacaacacacccaagggcagaactttgttacttaaacaccatcctgtttgcttctttcctcaggaactgtggctgcaccatctgtcttcatcttcccgccatctgatgagcagttgaaatctggaactgcctctgttgtgtgcctgctgaataacttctatcccagagaggccaaagtacagtggaaggtggataacgccctccaatcgggtaactcccaggagagtgtcacagagcaggacagcaaggacagcacctacagcctcagcagcaccctgacgctgagcaaagcagactacgagaaacacaaagtctacgcctgcgaagtcacccatcagggcctgagctcgcccgtcacaaagagcttcaacaggggagagtgttag

SEQ ID NO: 17 - protein, 364 aa, Artificial Sequence
  SIRPalphaD1 mutant-Fc (IMM01)
EEELQVIQPDKSVSVAAGESAILHCTVTSLIPVGPIQWFRGAGPARELIYNQKEGHFPRVTTVSESTKRENMDFSISISAITPADAGTYYCVKFRKGSPDTEFKSGAGTELSVRAKPSAPVVSGPAARATPQHEPKSCDKTHTCPPCPAPELLGGPSVFLFPPKPKDTLMISRTPEVTCVVVDVSHEDPEVKFNWYVDGVEVHNAKTKPREEQYNSTYRVVSVLTVLHQDWLNGKEYKCKVSNKALPAPIEKTISKAKGQPREPQVYTLPPSRDELTKNQVSLTCLVKGFYPSDIAVEWESNGQPENNYKTTPPVLDSDGSFFLYSKLTVDKSRWQQGNVFSCSVMHEALHNHYTQKSLSLSPG

SEQ ID NO: 18 - DNA, 57 bp, Artificial Sequence
  Signal peptide of murine IgG1 heavy chain
atgggatggtcatgtatcatcctttttctggtagcaactgcaactggagtacattca

SEQ ID NO: 19 - DNA, 9 bp, Artificial Sequence
  Kozak
gccgccacc

SEQ ID NO: 20 - protein, 471 aa, Artificial Sequence
  Cusatuzumab's heavy chain
MGWSCIILFLVATATGVHSEVQLVESGGGLVQPGGSLRLSCAASGFTFSVYYMNWVRQAPGKGLEWVSDINNEGGTTYYADSVKGRFTISRDNSKNSLYLQMNSLRAEDTAVYYCARDAGYSNHVPIFDSWGQGTLVTVSSASTKGPSVFPLAPSSKSTSGGTAALGCLVKDYFPEPVTVSWNSGALTSGVHTFPAVLQSSGLYSLSSVVTVPSSSLGTQTYICNVNHKPSNTKVDKKVEPKSCDKTHTCPPCPAPELLGGPSVFLFPPKPKDTLMISRTPEVTCVVVDVSHEDPEVKFNWYVDGVEVHNAKTKPREEQYNSTYRVVSVLTVLHQDWLNGKEYKCKVSNKALPAPIEKTISKAKGQPREPQVYTLPPSRDELTKNQVSLTCLVKGFYPSDIAVEWESNGQPENNYKTTPPVLDSDGSFFLYSKLTVDKSRWQQGNVFSCSVMHEALHNHYTQKSLSLSPGK

SEQ ID NO: 21 - protein, 235 aa, Artificial Sequence
  Cusatuzumab's light chain
MGWSCIILFLVATATGVHSQAVVTQEPSLTVSPGGTVTLTCGLKSGSVTSDNFPTWYQQTPGQAPRLLIYNTNTRHSGVPDRFSGSILGNKAALTITGAQADDEAEYFCALFISNPSVEFGGGTQLTVLGQPKAAPSVTLFPPSSEELQANKATLVCLISDFYPGAVTVAWKADSSPVKAGVETTTPSKQSNNKYAASSYLSLTPEQWKSHRSYSCQVTHEGSTVEKTVAPTECS

SEQ ID NO: 22 - protein, 406 aa, Artificial Sequence
  CD27(ECD)-Fc
ATPAPKSCPERHYWAQGKLCCQMCEPGTFLVKDCDQHRKAAQCDPCIPGVSFSPDHHTRPHCESCRHCNSGLLVRNCTITANAECACRNGWQCRDKECTECDPLPNPSLTARSSQALSPHPQPTHLPYVSEMLEARTAGHMQTLADFRQLPARTLSTHWPPQRSLCSSDFIREFEPKSCDKTHTCPPCPAPELLGGPSVFLFPPKPKDTLMISRTPEVTCVVVDVSHEDPEVKFNWYVDGVEVHNAKTKPREEQYNSTYRVVSVLTVLHQDWLNGKEYKCKVSNKALPAPIEKTISKAKGQPREPQVYTLPPSRDELTKNQVSLTCLVKGFYPSDIAVEWESNGQPENNYKTTPPVLDSDGSFFLYSKLTVDKSRWQQGNVFSCSVMHEALHNHYTQKSLSLSPGK

SEQ ID NO: 23 - protein, 397 aa, Artificial Sequence
  CD27-CAR
ATPAPKSCPERHYWAQGKLCCQMCEPGTFLVKDCDQHRKAAQCDPCIPGVSFSPDHHTRPHCESCRHCNSGLLVRNCTITANAECACRNGWQCRDKECTECDPLPNPSLTARSSQALSPHPQPTHLPYVSEMLEARTAGHMQTLADFRQLPARTLSTHWPPQRSLCSSDFIRTTTPAPRPPTPAPTIASQPLSLRPEACRPAAGGAVHTRGLDFACDFWVLVVVGGVLACYSLLVTVAFIIFWVRSKRSRLLHSDYMNMTPRRPGPTRKHYQPYAPPRDFAAYRSRVKFSRSAEPPAYQQGQNQLYNELNLGRREEYDVLDKRRGRDPEMGGKPRRKNPQEGLYNELQKDKMAEAYSEIGMKGERRRGKGHDGLYQGLSTATKDTYDALHMQALPPR